European Patent Application EP 4 497 819 A1, published January 29, 2025. Title: Genetically modified microorganisms and methods for production of 3-hydroxyadipate and/or 3-oxoadipate. Applicant: 東レ株式会社. Application JP. The sequence listing filed with the application follows.

SEQUENCE LISTING (61 sequences)

SEQ ID NO: 1 - protein, 405 aa, Escherichia coli
MPEPVAEPALNGLRLNLRIVSIVMFNFASYLTIGLPLAVLPGYVHDVMGFSAFWAGLVISLQYFATLLSRPHAGRYADSLGPKKIVVFGLCGCFLSGLGYLTAGLTASLPVISLLLLCLGRVILGIGQSFAGTGSTLWGVGVVGSLHIGRVISWNGIVTYGAMAMGAPLGVVFYHWGGLQALALIIMGVALVAILLAIPRPTVKASKGKPLPFRAVLGRVWLYGMALALASAGFGVIATFITLFYDAKGWDGAAFALTLFSCAFVGTRLLFPNGINRIGGLNVAMICFSVEIIGLLLVGVATMPWMAKIGVLLAGAGFSLVFPALGVVAVKAVPQQNQGAALATYTVFMDLSLGVTGPLAGLVMSWAGVPVIYLAAAGLVAIALLLTWRLKKRPPEHVPEAASSS

SEQ ID NO: 2 - DNA, 1218 bp, Escherichia coli
  source 1..1218: mol_type = genomic DNA
atgcccgaacccgtagccgaacccgcgctaaacggattgcgcctgaatttgcgcattgtctctatagtcatgtttaacttcgccagctacctcaccatcgggttgccgctcgctgtattaccgggctatgtccatgatgtgatgggctttagcgccttctgggcaggattggttatcagcctgcaatatttcgccaccttgctgagccgccctcatgccggacgttacgccgattcgctgggacccaaaaagattgtcgtcttcggtttatgcggctgctttttgagcggtctggggtatctgacggcaggattaaccgccagtctgcctgtcatcagcctgttattactttgcctggggcgcgtcatccttgggattgggcaaagttttgccggaacgggatcgaccctatggggcgttggcgtggttggctcgctgcatatcgggcgggtgatttcgtggaacggcattgtcacttacggggcgatggcgatgggtgcgccgttaggcgtcgtgttttatcactggggcggcttgcaggcgttagcgttaatcattatgggcgtggcgctggtggccattttgttggcgatcccgcgtccgacggtaaaagccagtaaaggcaaaccgctgccgtttcgcgcggtgcttgggcgcgtctggctgtacggtatggcgctggcactggcttccgccggatttggcgtcatcgccacctttatcacgctgttttatgacgctaaaggttgggacggtgcggctttcgcgctgacgctgtttagctgtgcgtttgtcggtacgcgtttgttattccctaacggcattaaccgtatcggtggcttaaacgtagcgatgatttgctttagcgttgagataatcggcctgctactggttggcgtggcgactatgccgtggatggcgaaaatcggcgtcttactggcgggggccgggttttcgctggtgttcccggcattgggtgtagtggcggtaaaagcggttccgcagcaaaatcagggggcggcgctggcaacttacaccgtatttatggatttatcgcttggcgtgactggaccactggctgggctggtgatgagctgggcgggcgtaccggtgatttatctggcggcggcgggactggtcgcaatcgcgttattactgacgtggcgattaaaaaaacggcctccggaacacgtccctgaggccgcctcatcatcttaa

SEQ ID NO: 3 - protein, 396 aa, Serratia grimesii
MTAISSKENNLQLNKRILSVVMFTFVCYLTIGLPLAVLPGFVHNDLGYNSVLAGLIISAQYFATLFSRPHAGRYADQLGPKKVVLFGLACCGVSGLFYAMAFWFTGLPLLSLILLCIGRVFLGVGESFASTGSTLWGIGLVGPLHTARVISWNGVATYGAMAAGAPLGVYLNQHWGLAGVAALIVLAVAVSLWLASAKPNVTIAAGKRIAFSAVLGRIWTYGLGLAMGTVGFGVIATFITLYYADKGWSGAAFSLTLFSVAFVGIRLIFSQTINRHGGLKVTLVSFLIEIIGLLLIWLATDPLMVQAGALLAGAGFSLVFPALGVEAVKQVPQQNQGTALGTYSAFLDLALGITGPLAGLLMSHMGVPSIYLAAALMVLMGALLTLRLLLQNRQNL

SEQ ID NO: 4 - DNA, 1191 bp, Serratia grimesii
  source 1..1191: mol_type = genomic DNA
atgaccgcaatcagctccaaagaaaacaatctccaactgaataaacgtattttatcggtcgtgatgttcaccttcgtttgttacctgaccatcggcttgccgttggcggtgctgccagggtttgtccataacgacctgggctacaactcggtgttggccggtttgatcattagtgcccagtatttcgctaccttgtttagccgaccgcatgccggtcgctatgccgatcagctcggaccgaaaaaagtggttttattcgggctggcttgttgcggtgtgagcggtctgttttatgccatggctttttggttcactggtctgccgttgctgagtttaattctgctgtgcattggcagggtgtttctcggcgtcggcgaaagctttgccagtacggggtctaccctatgggggattggcctggtggggccgttgcataccgcccgagttatctcatggaatggggtggcgacttacggtgcgatggctgccggggcaccgctcggtgtttacctcaatcagcactgggggttggccggggtggcggcgttgatcgtgctggcggtggcggtttcgctgtggctggcgagtgcgaagcccaacgtgacgatcgccgccggtaagcgcattgcctttagcgcagtgttggggcgtatttggacttacggtctgggactggcaatgggtaccgtggggtttggggtcatcgccacgtttatcaccctctactatgctgataaaggctggagcggggccgcgttctcactgacgctgttcagtgttgcctttgtcggtatccgcctgatatttagccagacgattaatcgccacggtggcttaaaagtcaccctagtgtcgttcctgattgagattatcgggttgttgttgatttggctggctacggacccgctaatggtgcaggccggagcgttgttggcaggtgccggtttctcgttggtgttcccggcgctgggcgtggaggcggtgaagcaagtgccacagcaaaatcagggcacagcactgggcacatactcggcatttctcgatctggcgttagggatcacggggccgttggctggtttgttaatgagccacatgggggtgccttcgatctatctggcggctgcgttgatggtgcttatgggcgctttgctgacgctgcgtttactgctgcaaaaccggcaaaatttatga

SEQ ID NO: 5 - DNA, 200 bp, Escherichia coli
  source 1..200: mol_type = genomic DNA
cgtaattgccctttaaaattcggggcgccgaccccatgtggtctcaagcccaaaggaagagtgaggcgagtcagtcgcgtaatgcttaggcacaggattgatttgtcgcaatgattgacacgattccgcttgacgctgcgtaaggtttttgtaattttacaggcaaccttttattcactaacaaatagctggtggaatat

SEQ ID NO: 6 - DNA, 30 bp, synthetic construct
  misc_feature 1..30: note = primer
  source 1..30: mol_type = other DNA
taccgtcgacctcgacgtaattgcccttta

SEQ ID NO: 7 - DNA, 41 bp, synthetic construct
  misc_feature 1..41: note = primer
  source 1..41: mol_type = other DNA
ggccccccctcgagtcattaagtactatattccaccagcta

SEQ ID NO: 8 - DNA, 774 bp, Pseudomonas putida
  source 1..774: mol_type = genomic DNA
atgccgcgatatatcgatgtgcaggcgcccgaacatggcgttcagctcattaccctgcaacggcccgaggccttgaatgccctgtgcaccgagctactggcagaactggccgctgcgctgcaggctgccgggaacgacgagcatgtccgtgccacagtgattaccggcagcgccaaggcattcgccgcaggcgccgacatccgcgagatggccgatcgcgacctggtcggcatcctcaatgacccgcgcgtagcgcattggcaaagcatcgccgcattcgccaaaccgctgattgctgcagtcaacggctatgccctgggtggcggttgcgaactggcaatgtgcgccgacatcgtcatcgccagtaccgacgcccgtttcggccagccggaaatcaaccttggcatcatccccggtgctggcggcacccagcgcctgttacgtgccgtcggtaagccgttggccatgcagatggtgctgacgggggaagccatcactgccctccgcgcccagcaggccggcctggtcagcgaaatcacccagcccgaactcaccgtagaacgcgccatgcaggttgcccgcagcatcgccgccaaagcgccgctggctgtgcgcctggccaaggaggcgttactgaaggccggtgataccgacctggccagcggcctgcgcttcgagcgccatgccttcaccctgctggcgggcaccgccgaccgcgatgaaggcatccgcgccttccaggaaaagcgccaggcccgcttccaagggcgctga

SEQ ID NO: 9 - DNA, 32 bp, synthetic construct
  misc_feature 1..32: note = primer
  source 1..32: mol_type = other DNA
ctggtggaatatatgcacgacgtattcatctg

SEQ ID NO: 10 - DNA, 41 bp, synthetic construct
  misc_feature 1..41: note = primer
  source 1..41: mol_type = other DNA
ctcgagtcattaagtgttaactcaaacccgctcgatggcca

SEQ ID NO: 11 - DNA, 696 bp, Pseudomonas putida
  source 1..696: mol_type = genomic DNA
ttgatcaataaaacgtacgagtccatcgccagcgcggtggaagggattaccgacggttcgaccatcatggtcggtggcttcggcacggctggcatgccgtccgagctgatcgatggcctcattgccaccggtgcccgcgacctgaccatcatcagcaacaacgccggcaacggcgagatcggcctggccgccctgctcatggcaggcagcgtgcgcaaggtggtctgctcgttcccgcgccagtccgactcctacgtgttcgacgaactgtaccgcgccggcaagatcgagctggaagtggtcccgcagggcaacctggccgagcgtatccgcgccgcaggctccggcattggtgcgttcttctcgccaaccggctacggcaccctgctggccgagggcaaggaaacccgtgagatcgatggccgcatgtacgtgctggaaatgccgctgcacgccgacttcgcactgatcaaggcgcacaagggtgaccgttggggcaacctgacctaccgcaaggccgcccgcaacttcggcccgatcatggccatggctgccaagaccgccatcgcccaggtcgaccaggtcgtcgaactcggtgaactggacccggaacacatcatcaccccgggtatcttcgtccagcgcgtggtcgccgtcaccggtgctgccgcttcttcgattgccaaagctgtctga

SEQ ID NO: 12 - DNA, 642 bp, Pseudomonas putida
  source 1..642: mol_type = genomic DNA
atgaccatcaccaaaaagctctcccgcaccgagatggcccaacgcgtggccgcagacatccaggaaggcgcgtacgtaaacctgggcatcggcgcaccgaccctggtggccaactacctgggcgacaaggaagtgttcctgcacagcgagaacggcctgctgggcatgggcccaagccctgcgccgggcgaggaagacgatgacctgatcaacgccggcaagcagcacgtcaccctgctgaccggtggtgccttcttccaccatgccgattcgttctcgatgatgcgtggcggccacctggacatcgctgtactgggcgccttccaggtgtcggtcaagggcgacctggccaactggcacacgggtgccgaaggctcgatcccggccgtaggcggtgcaatggacctggccaccggcgcccgccaggtgttcgtgatgatggaccacctgaccaagaccggcgaaagcaagctggtgcccgagtgcacctacccgctgaccggtatcgcttgcgtcagccgcatctacaccgacctggccgtactggaagtgacacctgaagggctgaaagtggtcgaaatctgcgcggacatcgactttgacgagctgcagaaactcagtggcgtgccgctgatcaagtga

SEQ ID NO: 13 - DNA, 55 bp, synthetic construct
  misc_feature 1..55: note = primer
  source 1..55: mol_type = other DNA
gagcgggtttgagttcaattgtagctggtggaatatttgatcaataaaacgtacg

SEQ ID NO: 14 - DNA, 34 bp, synthetic construct
  misc_feature 1..34: note = primer
  source 1..34: mol_type = other DNA
gagtcattaagtgtttcacttgatcagcggcacg

SEQ ID NO: 15 - protein, 509 aa, Serratia marcescens
MAESNAAIQSAAIIGAGTMGRGIAYLFAQKGIRTVLYNRNGNTLNQAREYIAQDLNKKVEQGKIALQDKGAVLANLMFTSVFEAIADSELVIETIAEQEQTKLEVLAAIAAVVKPDTLIATNTSSLSLNKLATAVTHSERFIGLHFFNPAPLMKLIEIIPAYFTAHATTERCRQLVAALGKHDVVCQATPGFIVNRMARPYYLEGFRLLEEHVARAAQIDRALKAGGRFRMGPLELTDFIGQDINYQVSRQIWQDMQYDPRYTPGHLQRSLVDAGLLGKKNGRSYFAAEETAPPVTAASNADVETLRVYGEHPFFTLLQQRAALQWPQLRVEQRPALPGLGSAVQINDAFTVSITDGRTASQLAEQTAADAFVVDVALNYADTTYLAAAHSRHASAANKALFLRLLHTAIPQVEFIKDSPALIVARVLSSLINESVIMVESGVCSREDIDVAAVAGVNYAGGIFDWLGKLGEKNVRTTLSNLAQLLHAARYAPHYTLLHAAQPALTTTP

SEQ ID NO: 16 - DNA, 1530 bp, Serratia marcescens
  source 1..1530: mol_type = genomic DNA
atggcagaaagtaatgcggcaattcaatcggctgcgattatcggcgcgggaacgatgggcagaggcatcgcttatcttttcgcgcaaaaaggcattcgcacggtgctttataatcgcaacggcaataccctcaatcaggctcgcgaatatatcgcgcaagacctgaacaagaaagtcgaacagggcaagatcgcgctgcaggataaaggcgcggtgctggccaatctaatgttcacttcagtgtttgaggccatcgccgacagcgagctggtgatagaaaccatcgccgagcaagaacaaaccaaacttgaggtgctggcggccatcgccgcggtggtcaagcccgacacgctgatcgccaccaatacctcctcactgtcgcttaacaagctggctactgcggtgacgcacagcgaacgctttatcggtttgcattttttcaaccccgcgccgctgatgaagctgattgaaatcattccggcctactttaccgcgcacgccaccaccgaacgctgccgccaactggtggcggcgttggggaaacacgatgtcgtctgccaggccacgccggggttcatcgtcaatcgcatggcccgcccctactacctggaagggttccgcctgttggaagaacacgtggcgcgcgcggctcagatcgaccgcgccctcaaggccggcgggcgcttccgcatggggccgctcgagctgaccgattttatcggccaagacatcaactatcaggtcagtcggcaaatctggcaggatatgcaatacgacccgcgctatacccccggtcatctgcagcgttcactggtcgatgccggtctgttggggaaaaagaacggccgctcctattttgccgccgaagaaaccgccccgccggtgacggccgccagcaatgcagacgtcgagacgctgcgcgtttacggcgagcaccctttttttaccctgttacagcagcgagccgcgcttcagtggccacagctgcgcgtggaacaacggccggcattaccggggctggggtcggccgtccagatcaatgacgctttcaccgtcagcatcaccgatggccgcacggcgagccaactggccgagcagacggcagcggatgcctttgtggtcgatgtcgccctgaactacgccgacacgacgtatctggcggcggcgcacagccgccacgcctctgcggccaataaggcgctgtttttacgcctgctgcacacggcaatcccgcaggttgaatttatcaaggactctccggcgcttatcgtcgcccgcgtcctcagcagcctgatcaatgagtcggtgatcatggtggaaagcggcgtctgcagccgggaagacatcgatgtcgccgccgtcgcgggcgttaactacgccggcggcattttcgactggctcggcaaactgggggagaaaaacgtcaggacaacgctgagcaatctggctcagctgctgcacgcggcgcgctatgcgccgcattacacccttctgcacgccgcgcaaccggcgctgacgaccacgccttaa

SEQ ID NO: 17 - DNA, 35 bp, synthetic construct
  misc_feature 1..35: note = primer
  source 1..35: mol_type = other DNA
ctggtggaatatagtactatggcagaaagtaatgc

SEQ ID NO: 18 - DNA, 39 bp, synthetic construct
  misc_feature 1..39: note = primer
  source 1..39: mol_type = other DNA
ttccaccagctaagtgctagcttaaggcgtggtcgtcag

SEQ ID NO: 19 - DNA, 35 bp, synthetic construct
  misc_feature 1..35: note = primer
  source 1..35: mol_type = other DNA
ccgccaagctcttcaacggaagatcacttcgcaga

SEQ ID NO: 20 - DNA, 35 bp, synthetic construct
  misc_feature 1..35: note = primer
  source 1..35: mol_type = other DNA
tcaggatgatctggagcctggggtgcctaatgagt

SEQ ID NO: 21 - DNA, 40 bp, synthetic construct
  misc_feature 1..40: note = primer
  source 1..40: mol_type = other DNA
cggccagtgaattcgagctctcgctccggcgacatatgca

SEQ ID NO: 22 - DNA, 35 bp, synthetic construct
  misc_feature 1..35: note = primer
  source 1..35: mol_type = other DNA
ctagaggatccccggatgataaagacactaacgct

SEQ ID NO: 23 - DNA, 70 bp, synthetic construct
  misc_feature 1..70: note = primer
  source 1..70: mol_type = other DNA
gtcagcacgtggtaaaaatgaaacactgttgtaaaaatgtggtgatcctcgtgtaggctggagctgcttc

SEQ ID NO: 24 - DNA, 70 bp, synthetic construct
  misc_feature 1..70: note = primer
  source 1..70: mol_type = other DNA
cgcagaccaccgcagaaaacatcattaatacgctggttattcagtaagttatgggaattagccatggtcc

SEQ ID NO: 25 - DNA, 18 bp, synthetic construct
  misc_feature 1..18: note = primer
  source 1..18: mol_type = other DNA
taagtgtagcgggagtca

SEQ ID NO: 26 - DNA, 18 bp, synthetic construct
  misc_feature 1..18: note = primer
  source 1..18: mol_type = other DNA
tcaactgctgaccatgca

SEQ ID NO: 27 - DNA, 20 bp, synthetic construct
  misc_feature 1..20: note = primer
  source 1..20: mol_type = other DNA
cggtgccctgaatgaactgc

SEQ ID NO: 28 - protein, 405 aa, Salmonella enterica
MPEPVAEPALNGLRLNLRIVSIVMFNFASYLTIGLPLAVLPGYVHDAMGFSAFWAGLIISLQYFATLLSRPHAGRYADVLGPKKIVVFGLCGCFLSGLGYLLADIASAWPMISLLLLGLGRVILGIGQSFAGTGSTLWGVGVVGSLHIGRVISWNGIVTYGAMAMGAPLGVLCYAWGGLQGLALTVMGVALLAVLLALPRPSVKANKGKPLPFRAVLGRVWLYGMALALASAGFGVIATFITLFYDAKGWDGAAFALTLFSVAFVGTRLLFPNGINRLGGLNVAMICFGVEIIGLLLVGTAAMPWMAKIGVLLTGMGFSLVFPALGVVAVKAVPPQNQGAALATYTVFMDMSLGVTGPLAGLVMTWAGVPVIYLAAAGLVAMALLLTWRLKKRPPSALPEAASSS

SEQ ID NO: 29 - protein, 406 aa, Klebsiella pneumoniae
MPEPVAEPALNGLRLNLRIVSVVIFNFASYLTIGLPLAVLPGYVHDVMGFSAFWAGLVISLQYFATLLSRPHAGRYADLLGPKKIVVFGLGGCFLSGLSYLLAAWGSGWPLISLLLLCLGRVILGIGQSFAGTGSTLWGVGVVGSLHIGRVISWNGIVTYGAMAMGAPLGVLCYSHIGLSGLAGVIMAVALVAILCALPRAAVKAAKGKAMSFRAVLGRVWPYGMALALASAGFGVIATFITLFYDAKGWDGAAFALTLFSCAFVGARLLFPNAINRLGGLNVAMLCFSVEAIGLLLVGFADTPMMAKIGTFLTGAGFSLVFPALGVVAVKAVPQHNQGSALATYTVFMDLSLGVSGPLAGLLMAWTGISMIYLAAAGLVMAALLLGWRLKKRPPVSEPEASAPGQ

SEQ ID NO: 30 - protein, 399 aa, Pectobacterium carotovorum
MPTPSPSEPALSGLRLNLRIVSIVAFNFASYLNIGLPLAVLPGYVHDHLGYSAFWAGLVISLQYFSTLLTRPHAGRSADEKGPKKIVVWGLAGVMLSGVFYLLAAFSDASPAITLLLLCLGRVVLGAGQSFAGTGATLWGVGVVGSRHIGRVISWNGIATYGAMAIGAPLGVWLNHIGGLKLLSVCIILIAAVAIVLALPRPTVQVAPGKKIPFREVLGKVWVYGIILAIASAGFGVIATFITLFYADRNWEGAALTLTIFSCAFVGARLVFPNSIQRFGGLRVAMACFVVEIVGLLLVWGAALPLMAEVGAFLAGAGFSLVFPALGVVAVQAVSPQNQGSALATYTIFLDLSLGIVGPVAGVLMAYTGIASIYLAAALLGLCGLALTWRLTQRTAVKE

SEQ ID NO: 31 - DNA, 1218 bp, Salmonella enterica
  source 1..1218: mol_type = genomic DNA
atgcccgaacccgtcgctgaaccggcgctaaacggattgcgcctcaatctgcgtattgtctccattgtgatgtttaactttgccagctacctgaccatcggcctgccgctcgccgtcttgcccggctatgtgcatgatgcgatgggattcagcgcgttctgggcggggcttattatcagcctgcaatacttcgccactctgttaagccgtccccatgccgggcggtatgcggatgtattagggccgaaaaaaatcgttgtctttggcttatgcggctgttttttaagcggactcggctacctgctggcggatatcgccagcgcctggccgatgatcagtttgttgctactggggctgggtcgcgtgattttggggattgggcaaagttttgccggcaccggttcgacactatggggcgtcggcgtcgtcgggtcgttgcatattggtcgggtcatctcctggaacggtatcgtcacctacggcgcaatggcgatgggcgcgccgctgggcgtgctgtgttatgcctggggcgggttacagggactggcgctaacggtgatgggcgtggcgctgttggcggtactgttagcccttccacgtccgtcggtgaaggcgaacaaaggcaagccgctgccgtttcgcgcggtgctggggcgtgtctggctgtatggtatggcgttggcgctggcctcggcagggtttggcgtcatcgcgacgtttattaccttattttatgatgctaaaggttgggatggcgccgcctttgcgctcacgttatttagcgtcgcgtttgtcggcacgcgtttgctgttccctaacggtatcaatcgcttaggcgggttgaatgtcgccatgatctgctttggcgtggagattattggtctgttactggtggggacggcagccatgccgtggatggcaaaaatcggcgttttactcacggggatggggttttcgctggtctttccggcgctgggtgtggtggccgtcaaagccgtgccgccgcagaaccagggcgcggcgctggcgacctataccgtctttatggatatgtctttgggggtgaccgggccgctggcggggctggtgatgacctgggcgggcgtgccggtgatttatctggcggcggccgggctggtagcgatggcgctattactgacctggcgcttaaaaaaacggcctccgtctgcactgccggaggccgcatcatcgtcgtga

SEQ ID NO: 32 - DNA, 1221 bp, Klebsiella pneumoniae
  source 1..1221: mol_type = genomic DNA
atgcccgaacccgtcgccgaaccggcgcttaatggactgcgcctcaatctgcggattgtctctgtcgttatctttaactttgccagctacctcaccatcggcctgccgctggcggtgctgcccggctatgttcatgatgtcatgggctttagcgctttctgggccgggctggtgattagcctgcaatatttcgccacgctgctcagccgcccgcatgccgggcgctatgccgacctgctggggcccaaaaagattgtcgtcttcggcctcggcggctgctttttgagcggtttgagctatctgctggccgcctggggcagcggctggccactgattagcctgctgctgttatgcctcggacgggtgatccttggtatcggccagagcttcgccggcacaggctcgacgctgtggggcgtcggcgtggtcggttcgctgcatatcgggcgggtgatctcgtggaacgggattgtgacctatggggcgatggcgatgggcgcgccgctcggcgtgctgtgctattcgcacattggcctcagcggtctggccggggtcattatggcggtagcgctggtggctatcctctgcgcgctgccccgcgcggcggtgaaggctgccaaaggcaaagcgatgtcgtttcgcgcggtgctcggccgggtctggccctacggcatggcgctggcgttggcctccgccggctttggggtgatcgccacctttatcacgctattttatgacgccaaaggttgggacggcgcggctttcgcgctgacattattcagctgcgcgttcgttggcgcgcggctgctgtttcccaacgccattaaccgactcggcgggctgaacgtggcgatgctctgctttagcgtggaggcgatcggcctgctgctggtcggctttgccgatacgccgatgatggcgaaaatcggtactttccttaccggggctggcttttcgctggtctttccggcgctgggggtggtggcggtgaaagcggtgccgcagcacaatcaggggtcggcgctggcgacctataccgtgtttatggatttgtcgttgggcgtcagcgggccgctggccggattgctgatggcgtggaccgggatctcgatgatttatctcgccgcggcggggctggtgatggcggcgctgctgttgggctggcggctaaaaaaacggcccccggttagcgaaccggaggccagcgcaccaggccagtaa

SEQ ID NO: 33 - DNA, 1200 bp, Pectobacterium carotovorum
  source 1..1200: mol_type = genomic DNA
atgccaacaccttccccatccgaaccggcgctgagcggtctgcgccttaatctgcgcatcgtttcaattgtggcgttcaacttcgccagctatctgaatattggcctgccgttggcggtgttgccggggtatgtgcatgaccaccttggctatagcgcgttctgggccggtctggtgatcagcctgcaatatttttccacgttgttgacccgcccgcacgcggggcgtagcgccgatgaaaaaggaccgaaaaaaatcgtcgtttgggggctggctggcgtcatgctgagcggggtgttttacctgctggccgcttttagtgatgcatcgcccgcgatcacgctgctgctactgtgtctcgggcgcgttgtgctgggggctgggcagagttttgccgggacaggtgcaacgctctggggcgttggtgtggtcggttcccgacacatcgggcgtgtgatttcatggaatggcattgccacttacggcgcgatggcgattggcgcaccgctcggcgtctggctcaaccatatcggtgggctaaaactgctctccgtgtgcataatcctgattgcggcggtggcgattgttctcgcgctgccgcgcccgacggtgcaggtcgcgccggggaaaaagattcccttccgcgaagtgctggggaaagtctgggtttacggcattattctggcaatcgcctcagcaggttttggcgtgatcgccacctttatcacgctgttttatgccgataggaactgggaaggtgccgcgctgacgctgacgattttcagctgcgcttttgtcggtgcgcgattggtgtttcctaacagcattcagcggtttggtggattgcgcgtagcgatggcgtgctttgtggttgagatcgtggggttattgctggtgtggggggcggcgctgccgttgatggccgaagtcggcgcattcctcgcgggggcgggtttctctttggtgttcccggcattaggcgtggttgccgttcaggctgtctcgccgcagaatcagggcagcgcactggcgacctatacgatatttctcgatttgtcgctgggcatcgtcgggccagtggcgggtgtgctgatggcctataccggtatcgcctctatttatctggcggcggcgttgctggggctatgtggtctggcgctgacgtggcggctgactcagcgcacggcagtcaaagaataa

SEQ ID NO: 34 - DNA, 34 bp, synthetic construct
  misc_feature 1..34: note = primer
  source 1..34: mol_type = other DNA
cggccagtgaattcgtcgctccggcgacatatgc

SEQ ID NO: 35 - DNA, 34 bp, synthetic construct
  misc_feature 1..34: note = primer
  source 1..34: mol_type = other DNA
gttggtaccgagctcgaggatcaccacattttta

SEQ ID NO: 36 - DNA, 34 bp, synthetic construct
  misc_feature 1..34: note = primer
  source 1..34: mol_type = other DNA
ctcgagctcggtaccaacttactgaataaccagc

SEQ ID NO: 37 - DNA, 35 bp, synthetic construct; identical to SEQ ID NO: 22
  misc_feature 1..35: note = primer
  source 1..35: mol_type = other DNA

SEQ ID NO: 38 - DNA, 34 bp, synthetic construct
  misc_feature 1..34: note = primer
  source 1..34: mol_type = other DNA
atgtggtgatcctcgatgcccgaacccgtcgctg

SEQ ID NO: 39 - DNA, 46 bp, synthetic construct
  misc_feature 1..46: note = primer
  source 1..46: mol_type = other DNA
ttattcagtaagttggtaccgagctctcacgacgatgatgcggcct

SEQ ID NO: 40 - DNA, 34 bp, synthetic construct
  misc_feature 1..34: note = primer
  source 1..34: mol_type = other DNA
atgtggtgatcctcgatgcccgaacccgtcgccg

SEQ ID NO: 41 - DNA, 46 bp, synthetic construct
  misc_feature 1..46: note = primer
  source 1..46: mol_type = other DNA
ttattcagtaagttggtaccgagctcttactggcctggtgcgctgg

SEQ ID NO: 42 - DNA, 34 bp, synthetic construct
  misc_feature 1..34: note = primer
  source 1..34: mol_type = other DNA
atgtggtgatcctcgatgccaacaccttccccat

SEQ ID NO: 43 - DNA, 46 bp, synthetic construct
  misc_feature 1..46: note = primer
  source 1..46: mol_type = other DNA
ttattcagtaagttggtaccgagctcttattctttgactgccgtgc

SEQ ID NO: 44 - DNA, 34 bp, synthetic construct
  misc_feature 1..34: note = primer
  source 1..34: mol_type = other DNA
atgtggtgatcctcgatgaccgcaatcagctcca

SEQ ID NO: 45 - DNA, 46 bp, synthetic construct
  misc_feature 1..46: note = primer
  source 1..46: mol_type = other DNA
ttattcagtaagttggtaccgagctctcataaattttgccggtttt

SEQ ID NO: 46 - protein, 471 aa, Escherichia coli
MTDLPDSTRWQLWIVAFGFFMQSLDTTIVNTALPSMAQSLGESPLHMHMVIVSYVLTVAVMLPASGWLADKVGVRNIFFTAIVLFTLGSLFCALSGTLNELLLARALQGVGGAMMVPVGRLTVMKIVPREQYMAAMTFVTLPGQVGPLLGPALGGLLVEYASWHWIFLINIPVGIIGAIATLLLMPNYTMQTRRFDLSGFLLLAVGMAVLTLALDGSKGTGLSPLTIAGLVAVGVVALVLYLLHARNNNRALFSLKLFRTRTFSLGLAGSFAGRIGSGMLPFMTPVFLQIGLGFSPFHAGLMMIPMVLGSMGMKRIVVQVVNRFGYRRVLVATTLGLSLVTLLFMTTALLGWYYVLPFVLFLQGMVNSTRFSSMNTLTLKDLPDNLASSGNSLLSMIMQLSMSIGVTIAGLLLGLFGSQHVSVDSGTTQTVFMYTWLSMALIIALPAFIFARVPNDTHQNVAISRRKRSAQ

SEQ ID NO: 47 - DNA, 1416 bp, Escherichia coli
  source 1..1416: mol_type = genomic DNA
atgacagatcttcccgacagcacccgttggcaattgtggattgtggctttcggcttctttatgcagtcgctggacaccaccatcgtaaacaccgcccttccctcaatggcgcaaagcctcggggaaagtccgttgcatatgcacatggtcattgtctcttatgtgctgaccgtggcggtgatgctgcccgccagcggctggctggcggacaaagtcggcgtgcgcaatattttctttaccgccatcgtgctgtttactctcggttcactgttttgcgcgctttccggcacgctgaacgaactgttgctggcacgcgcgttacagggcgttggcggcgcgatgatggtgccggtcggcagattgacggtgatgaaaatcgtaccgcgcgagcaatatatggcggcgatgacctttgtcacgttacccggtcaggtcggtccgctgctcggtccggcgctcggcggtctgctggtggagtacgcatcgtggcactggatctttttgatcaacattccggtggggattatcggtgcgatcgccacattgctgttaatgccgaactacaccatgcagacgcggcgctttgatctctccggatttttattgctggcggttggcatggcggtattaaccctggcgctggacggcagtaaaggtacaggtttatcgccgctgacgattgcaggcctggtcgcagttggcgtggtggcactggtgctttatctgctgcacgccagaaataacaaccgtgccctgttcagtctgaaactgttccgtactcgtaccttttcgctgggcctggcggggagctttgccggacgtattggcagtggcatgttgccctttatgacaccggttttcctgcaaattggcctcggtttctcgccgtttcatgccggactgatgatgatcccgatggtgcttggcagcatgggaatgaagcgaattgtggtacaggtggtgaatcgctttggttatcgtcgggtactggtagcgaccacgctgggtctgtcgctggtcaccctgttgtttatgactaccgccctgctgggctggtactacgttttgccgttcgtcctgtttttacaagggatggtcaactcgacgcgtttctcctccatgaacaccctgacgctgaaagatctcccggacaatctggcgagcagcggcaacagcctgctgtcgatgattatgcaattgtcgatgagtatcggcgtcactatcgccgggctgttgctgggactttttggttcacagcatgtcagcgtcgacagcggcaccacacaaaccgtctttatgtacacctggcttagcatggcgttgatcatcgcccttccggcgttcatctttgccagagtgccgaacgatacgcatcaaaatgtagctatttcgcggcgaaaaaggagcgcgcaatga

SEQ ID NO: 48 - protein, 206 aa, Escherichia coli
MTLEWWFAYLLTSIILSLSPGSGAINTMTTSLNHGYRGAVASIAGLQTGLAIHIVLVGVGLGTLFSRSVIAFEVLKWAGAAYLIWLGIQQWRAAGAIDLKSLASTQSRRHLFQRAVFVNLTNPKSIVFLAALFPQFIMPQQPQLMQYIVLGVTTIVVDIIVMIGYATLAQRIALWIKGPKQMKALNKIFGSLFMLVGALLASARHA

SEQ ID NO: 49 - DNA, 621 bp, Escherichia coli
  source 1..621: mol_type = genomic DNA
atgaccttagaatggtggtttgcctacctgctgacatcgatcattttaagcctgtcgccaggctctggtgcaatcaacactatgaccacctcgctcaaccacggttatcgcggcgcggtggcgtctattgctgggcttcagaccggactggcgattcatattgtgctggttggcgtggggttggggacgctattttcccgctcagtgattgcgtttgaagtgttgaagtgggcaggcgcggcttacttgatttggctgggaatccagcagtggcgcgccgctggtgcaattgaccttaaatcgctggcctctactcaatcgcgtcgacatttgttccagcgcgcagtttttgtgaatctcaccaatcccaaaagtattgtgtttctggcggcgctatttccgcaattcatcatgccgcaacagccgcaactgatgcagtatatcgtgctcggcgtcaccactattgtggtcgatattattgtgatgatcggttacgccacccttgctcaacggattgctctatggattaaaggaccaaagcagatgaaggcgctgaataagattttcggctcgttgtttatgctggtgggagcgctgttagcatcggcgaggcatgcgtga

SEQ ID NO: 50 - protein, 344 aa, Aspergillus oryzae
MAVENAIPTTSSTDAQALPDEPKPAKKGYGWRFWAIFPGLCELYVWVINGYFVSQTAVQPLYGQVANIFGRRWPTILSVALFALGSGLGGGASSTEMLIARSLLPTWCLPVYFQLVLEATPKKSGIDLFASFIPMVPGAIVGGVLITVTGKDKPLLVAGFILMAVGMGLFTMLDDRTNTVRWVIYQVILALGSVISLIATLPAVLASLPESDVATATATWAFLRSFGSIWCVSIPSAVFNSRFTDLVGRIASPQLRGVLLGGGAYQLATKAFMESLDDTPVVKAQVVSVYVDSLKLVWQVGIAFAALGVPLSLLIRSLALRDELNAEFGLEETRTENVEEVRVQ

SEQ ID NO: 51 - DNA, 1035 bp, Aspergillus oryzae
  source 1..1035: mol_type = genomic DNA
atggctgttgagaatgccataccgacaacgagcagcaccgatgcccaagccctcccagacgagccgaagcctgccaaaaagggctatggatggcggttctgggccatcttccccggtctatgcgaactatacgtctgggtaatcaacgggtacttcgtcagccaaaccgccgttcagcctttatacggccaagttgccaatatctttggccgccgatggccgaccatcctctccgtggctctcttcgccttgggaagtggtctcggcggtggcgcatcgagtacggagatgctcattgcgagatcattgttgccaacctggtgcctccccgtctacttccaattggtcctcgaagccacgcccaagaaatccggcattgacctattcgcctccttcatccccatggtccccggcgccatcgtcggcggagtcctcatcaccgtcacaggcaaagacaagccgctcctcgtcgccgggttcatcctcatggccgtcggaatgggcctgttcaccatgctcgatgaccgcaccaacaccgtccgctgggtcatctaccaagtgatactagctcttggctctgtcatttccctcatcgccacacttcccgctgttctggccagtttgcccgagtccgatgtcgcgactgctacggctacctgggcgtttctgcgtagttttggttccatttggtgtgtttcgattccctcggcggtttttaattcgaggtttacggacctcgtgggtcgtattgctagtccacagttgcggggcgttcttttgggtggtggtgcgtatcaacttgctactaaagcttttatggaatcgctggatgatacgcctgtggttaaggcgcaggtggtgagcgtgtatgtggatagcttgaagcttgtgtggcaggttggcattgcttttgctgcgcttggggtgcctttgtctttgctgattcggagtcttgcgttacgcgatgagttgaatgccgagtttgggcttgaggagacaaggacagagaatgtcgaggaggttagggtgcagtga

SEQ ID NO: 52 - DNA, 34 bp, synthetic construct
  misc_feature 1..34: note = primer
  source 1..34: mol_type = other DNA
atgtggtgatcctcgatgacagatcttcccgaca

SEQ ID NO: 53 - DNA, 46 bp, synthetic construct
  misc_feature 1..46: note = primer
  source 1..46: mol_type = other DNA
ttattcagtaagttggtaccgagctctcattgcgcgctcctttttc

SEQ ID NO: 54 - DNA, 34 bp, synthetic construct
  misc_feature 1..34: note = primer
  source 1..34: mol_type = other DNA
atgtggtgatcctcgatgaccttagaatggtggt

SEQ ID NO: 55 - DNA, 46 bp, synthetic construct
  misc_feature 1..46: note = primer
  source 1..46: mol_type = other DNA
ttattcagtaagttggtaccgagctctcacgcatgcctcgccgatg

SEQ ID NO: 56 - DNA, 34 bp, synthetic construct
  misc_feature 1..34: note = primer
  source 1..34: mol_type = other DNA
atgtggtgatcctcgatggctgttgagaatgcca

SEQ ID NO: 57 - DNA, 46 bp, synthetic construct
  misc_feature 1..46: note = primer
  source 1..46: mol_type = other DNA
ttattcagtaagttggtaccgagctctcactgcaccctaacctcct

SEQ ID NO: 58 - protein, 394 aa, Escherichia coli
MKRQRNVNLLLMLVLLVAVGQMAQTIYIPAIADMARDLNVREGAVQSVMGAYLLTYGVSQLFYGPISDRVGRRPVILVGMSIFMLATLVAVTTSSLTVLIAASAMQGMGTGVGGVMARTLPRDLYERTQLRHANSLLNMGILVSPLLAPLIGGLLDTMWNWRACYLFLLVLCAGVTFSMARWMPETRPVDAPRTRLLTSYKTLFGNSGFNCYLLMLIGGLAGIAAFEACSGVLMGAVLGLSSMTVSILFILPIPAAFFGAWFAGRPNKRFSTLMWQSVICCLLAGLLMWIPDWFGVMNVWTLLVPAALFFFGAGMLFPLATSGAMEPFPFLAGTAGALVGGLQNIGSGVLASLSAMLPQTGQGSLGLLMTLMGLLIVLCWLPLATRMSHQGQPV

SEQ ID NO: 59 - DNA, 1185 bp, Escherichia coli
  source 1..1185: mol_type = genomic DNA
atgaaaaggcaaagaaacgtcaatttgttattgatgttggtattactcgtggccgtcggtcagatggcgcaaaccatttatattccagctattgccgatatggcgcgcgatctcaacgtccgtgaaggggcggtgcagagcgtaatgggcgcttatctgctgacttacggtgtctcacagctgttttatggcccgatttccgaccgcgtgggccgccgaccggtgatcctcgtcggaatgtccatttttatgctggcaacgctggtcgcggtcacgacctccagtttgacggtgttgattgccgccagcgcgatgcaggggatgggcaccggcgttggcggcgtaatggcgcgtactttaccgcgagatttatatgaacggacacagttgcgccatgctaacagcctgttaaacatggggattctcgtcagtccgttgctcgcaccgctaatcggcggtctgctggatacgatgtggaactggcgcgcctgttatctctttttgttggttctttgtgctggtgtgaccttcagtatggcccgctggatgccggaaacgcgtccggtcgatgcaccgcgcacgcgcctgcttaccagttataaaacgcttttcggtaacagcggttttaactgttatttgctgatgctgattggcggtctggccgggattgccgcctttgaagcctgctccggcgtgctgatgggcgcggtgttagggctgagcagtatgacggtcagtattttgtttattctgccgattccggcagcgttttttggcgcatggtttgccggacgtcccaataaacgcttctccacgttaatgtggcagtcggttatctgctgcctgctggctggcttgctgatgtggatccccgactggtttggcgtgatgaatgtctggacgctgctcgttcccgccgcgctgttctttttcggtgccgggatgctgtttccgctggcgaccagcggcgcgatggagccgttccccttcctggcgggcacggctggcgcgctggtcggcggtctgcaaaacattggttccggcgtgctggcgtcgctctctgcgatgttgccgcaaaccggtcagggcagcctggggttgttgatgaccttaatgggattgttgatcgtgctgtgctggctgccgctggcgacgcggatgtcgcatcaggggcagcccgtttaa

SEQ ID NO: 60 - DNA, 34 bp, synthetic construct
  misc_feature 1..34: note = primer
  source 1..34: mol_type = other DNA
atgtggtgatcctcgatgaaaaggcaaagaaacg

SEQ ID NO: 61 - DNA, 46 bp, synthetic construct
  misc_feature 1..46: note = primer
  source 1..46: mol_type = other DNA
ttattcagtaagttggtaccgagctcttaaacgggctgcccctgat